European Patent Application EP 4 174 491 A1, published May 3, 2023. Title: COMPOSITIONS AND METHODS FOR DETECTING PYROPHOSPHATE PRODUCTS OF ENZYME REACTIONS USING PYRIDYLAZOANILINE DYES. Applicant: New England Biolabs, Inc. Application Not yet assigned. The sequence listing filed with the application follows.

SEQUENCE LISTING (13 sequences)

SEQ ID NO: 1 - DNA, 20 bp, Artificial Sequence
  Synthetic construct
cctgctctgccgcttcacgc

SEQ ID NO: 2 - DNA, 28 bp, Artificial Sequence
  Synthetic construct
tccggataaaaacgtcgatgacatttgc

SEQ ID NO: 3 - DNA, 28 bp, Artificial Sequence
  Synthetic construct
gatgacgcatcctcacgataatatccgg

SEQ ID NO: 4 - DNA, 24 bp, Artificial Sequence
  Synthetic construct
ccatgattcagtgtgcccgtctgg

SEQ ID NO: 5 - DNA, 23 bp, Artificial Sequence
  Synthetic construct
cgaacgtcgcgcagagaaacagg

SEQ ID NO: 6 - DNA, 26 bp, Artificial Sequence
  Synthetic construct
cctggatccagatgcagtaataccgc

SEQ ID NO: 7 - DNA, 22 bp, Artificial Sequence
  Synthetic construct
tccgaggatggtattcgtcatg

SEQ ID NO: 8 - DNA, 24 bp, Artificial Sequence
  Synthetic construct
ggggcaccttctccaactcatact

SEQ ID NO: 9 - DNA, 24 bp, Artificial Sequence
  Synthetic construct
cgagctaccacgcagacatcaacc

SEQ ID NO: 10 - DNA, 24 bp, Artificial Sequence
  Synthetic construct
ggggcaccttctccaactcatact

SEQ ID NO: 11 - DNA, 23 bp, Artificial Sequence
  Synthetic construct
cctcatttggggaggggttatct

SEQ ID NO: 12 - DNA, 20 bp, Artificial Sequence
  Synthetic construct
gaagagccaaggacaggtac

SEQ ID NO: 13 - DNA, 20 bp, Artificial Sequence
  Synthetic construct
cctccaaatcaagcctctac